European Patent Specification EP 4 036 101 B1, published September 2, 2026. Title: MODIFIED OLIGOMERIC COMPOUNDS COMPRISING TRICYCLO-DNA NUCLEOSIDES AND USES THEREOF. Applicant: Synthena AG. The sequence listing filed with the application follows.

SEQUENCE LISTING (47 sequences)

SEQ ID NO: 1 - DNA, 13 bp, Artificial Sequence
  Synthetic
  misc_feature (1)..(13): deoxyribonucleoside with tricyclic sugar
  modified_base (1)..(2): m5c
  modified_base (4)..(4): m5c
  modified_base (7)..(7): m5c
  modified_base (11)..(12): m5c
cctcggcttacct

SEQ ID NO: 2 - DNA, 13 bp, Artificial Sequence
  Synthetic
  misc_feature (1)..(13): deoxyribonucleoside with tricyclic sugar
  modified_base (2)..(3): m5c
  modified_base (5)..(5): m5c
  modified_base (8)..(8): m5c
  modified_base (12)..(13): m5c
acctcggcttacc

SEQ ID NO: 3 - DNA, 13 bp, Artificial Sequence
  Synthetic
  misc_feature (1)..(2): deoxyribonucleoside with tricyclic sugar
  modified_base (1)..(2): m5c
  misc_feature (3)..(3): 2'-modified ribonucleoside, preferably 2'-O-methyl ribonucleoside
  modified_base (4)..(4): m5c
  misc_feature (4)..(13): deoxyribonucleoside with tricyclic sugar
  modified_base (7)..(7): m5c
  modified_base (11)..(12): m5c
ccucggcttacct

SEQ ID NO: 4 - DNA, 15 bp, Artificial Sequence
  Synthetic
  misc_feature (1)..(4): deoxyribonucleoside with tricyclic sugar
  misc_feature (5)..(5): 2'-modified ribonucleoside, preferably 2'-O-methyl ribonucleoside
  misc_feature (6)..(15): deoxyribonucleoside with tricyclic sugar
  modified_base (8)..(8): m5c
  modified_base (13)..(13): m5c
aagauggcatttcta

SEQ ID NO: 5 - DNA, 15 bp, Artificial Sequence
  Synthetic
  misc_feature (1)..(7): deoxyribonucleoside with tricyclic sugar
  modified_base (1)..(1): m5c
  modified_base (4)..(5): m5c
  misc_feature (8)..(8): 2'-modified ribonucleoside, preferably 2'-O-methyl ribonucleoside
  misc_feature (9)..(15): deoxyribonucleoside with tricyclic sugar
  modified_base (13)..(14): m5c
catcctggagttcct

SEQ ID NO: 6 - DNA, 15 bp, Artificial Sequence
  Synthetic
  misc_feature (1)..(9): deoxyribonucleoside with tricyclic sugar
  modified_base (2)..(3): m5c
  modified_base (6)..(7): m5c
  misc_feature (10)..(10): 2'-modified ribonucleoside, preferably 2'-O-methyl ribonucleoside
  misc_feature (11)..(15): deoxyribonucleoside with tricyclic sugar
  modified_base (15)..(15): m5c
gccatcctggagttc

SEQ ID NO: 7 - DNA, 15 bp, Artificial Sequence
  Synthetic
  misc_feature (1)..(15): deoxyribonucleoside with tricyclic sugar
  modified_base (1)..(2): m5c
  modified_base (4)..(4): m5c
  modified_base (7)..(9): m5c
  modified_base (14)..(15): m5c
ccgctgcccaatgcc

SEQ ID NO: 8 - DNA, 15 bp, Artificial Sequence
  Synthetic
  misc_feature (1)..(4): deoxyribonucleoside with tricyclic sugar
  modified_base (2)..(2): m5c
  misc_feature (5)..(5): 2'-modified ribonucleoside, preferably 2'-O-methyl ribonucleoside
  misc_feature (6)..(15): deoxyribonucleoside with tricyclic sugar
  modified_base (8)..(10): m5c
  modified_base (12)..(12): m5c
acttcatcccactga

SEQ ID NO: 9 - DNA, 15 bp, Artificial Sequence
  Synthetic
  misc_feature (1)..(15): deoxyribonucleoside with tricyclic sugar
  modified_base (5)..(5): m5c
  modified_base (9)..(9): m5c
  modified_base (12)..(12): m5c
atttcattcaactgt

SEQ ID NO: 10 - DNA, 15 bp, Artificial Sequence
  Synthetic
  misc_feature (1)..(15): deoxyribonucleoside with tricyclic sugar
  modified_base (1)..(1): m5c
  modified_base (9)..(10): m5c
ctggagttcctgtaa

SEQ ID NO: 11 - DNA, 15 bp, Artificial Sequence
  Synthetic
  misc_feature (1)..(3): deoxyribonucleoside with tricyclic sugar
  modified_base (1)..(1): m5c
  misc_feature (4)..(4): 2'-modified ribonucleoside, preferably 2'-O-methyl ribonucleoside
  misc_feature (5)..(15): deoxyribonucleoside with tricyclic sugar
  modified_base (9)..(10): m5c
ctggagttcctgtaa

SEQ ID NO: 12 - DNA, 15 bp, Artificial Sequence
  Synthetic
  misc_feature (1)..(5): deoxyribonucleoside with tricyclic sugar
  modified_base (2)..(3): m5c
  misc_feature (6)..(6): 2'-modified ribonucleoside, preferably 2'-O-methyl ribonucleoside
  misc_feature (7)..(15): deoxyribonucleoside with tricyclic sugar
  modified_base (11)..(12): m5c
tcctggagttcctgt

SEQ ID NO: 13 - DNA, 15 bp, Artificial Sequence
  Synthetic
  misc_feature (1)..(10): deoxyribonucleoside with tricyclic sugar
  modified_base (6)..(6): m5c
  misc_feature (11)..(11): 2'-modified ribonucleoside, preferably 2'-O-methyl ribonucleoside
  misc_feature (12)..(15): deoxyribonucleoside with tricyclic sugar
  modified_base (12)..(12): m5c
  modified_base (15)..(15): m5c
gtgttcttgtacttc

SEQ ID NO: 14 - DNA, 15 bp, Artificial Sequence
  Synthetic
  misc_feature (1)..(4): deoxyribonucleoside with tricyclic sugar
  modified_base (1)..(1): m5c
  misc_feature (5)..(5): 2'-modified ribonucleoside, preferably 2'-O-methyl ribonucleoside
  misc_feature (6)..(15): deoxyribonucleoside with tricyclic sugar
  modified_base (12)..(12): m5c
ctgaaggtgttcttg

SEQ ID NO: 15 - DNA, 15 bp, Artificial Sequence
  Synthetic
  misc_feature (1)..(8): deoxyribonucleoside with tricyclic sugar
  modified_base (1)..(1): m5c
  modified_base (3)..(4): m5c
  misc_feature (9)..(9): 2'-modified ribonucleoside, preferably 2'-O-methyl ribonucleoside
  misc_feature (10)..(15): deoxyribonucleoside with tricyclic sugar
ctccggttctgaagg

SEQ ID NO: 16 - DNA, 15 bp, Artificial Sequence
  Synthetic
  misc_feature (1)..(9): deoxyribonucleoside with tricyclic sugar
  modified_base (7)..(8): m5c
  misc_feature (10)..(10): 2'-modified ribonucleoside, preferably 2'-O-methyl ribonucleoside
  misc_feature (11)..(15): deoxyribonucleoside with tricyclic sugar
  modified_base (14)..(14): m5c
ttgaatcctutaaca

SEQ ID NO: 17 - DNA, 15 bp, Artificial Sequence
  Synthetic
  misc_feature (1)..(5): deoxyribonucleoside with tricyclic sugar
  modified_base (1)..(1): m5c
  modified_base (5)..(5): m5c
  misc_feature (6)..(6): 2'-modified ribonucleoside, preferably 2'-O-methyl ribonucleoside
  misc_feature (7)..(15): deoxyribonucleoside with tricyclic sugar
  modified_base (12)..(12): m5c
ctttcataatgctgg

SEQ ID NO: 18 - DNA, 15 bp, Artificial Sequence
  Synthetic
  misc_feature (1)..(9): deoxyribonucleoside with tricyclic sugar
  modified_base (1)..(1): m5c
  modified_base (5)..(5): m5c
  misc_feature (10)..(10): 2'-modified ribonucleoside, preferably 2'-O-methyl ribonucleoside
  misc_feature (11)..(15): deoxyribonucleoside with tricyclic sugar
  modified_base (12)..(12): m5c
ctttcataaugctgg

SEQ ID NO: 19 - DNA, 15 bp, Artificial Sequence
  Synthetic
  misc_feature (1)..(15): deoxyribonucleoside with tricyclic sugar
  modified_base (8)..(8): m5c
  modified_base (13)..(13): m5c
aagatggcatttcta

SEQ ID NO: 20 - DNA, 18 bp, Artificial Sequence
  Synthetic
  misc_feature (1)..(5): deoxyribonucleoside with tricyclic sugar
  modified_base (1)..(1): m5c
  modified_base (4)..(4): m5c
  misc_feature (6)..(6): 2'-modified ribonucleoside, preferably 2'-O-methyl ribonucleoside
  misc_feature (7)..(18): deoxyribonucleoside with tricyclic sugar
  modified_base (7)..(7): m5c
  modified_base (10)..(10): m5c
  modified_base (13)..(13): m5c
  modified_base (16)..(16): m5c
cagcagcagcagcagcag

SEQ ID NO: 21 - DNA, 15 bp, Artificial Sequence
  Synthetic
  misc_feature (1)..(15): deoxyribonucleoside with tricyclic sugar
  modified_base (2)..(3): m5c
  modified_base (8)..(8): m5c
  modified_base (11)..(11): m5c
  modified_base (13)..(14): m5c
gcctggacagctcct

SEQ ID NO: 22 - DNA, 15 bp, Artificial Sequence
  Synthetic
  misc_feature (1)..(4): deoxyribonucleoside with tricyclic sugar
  misc_feature (6)..(15): deoxyribonucleoside with tricyclic sugar
  modified_base (8)..(8): m5c
  modified_base (13)..(13): m5c
aagatggcatttcta

SEQ ID NO: 23 - DNA, 13 bp, Artificial Sequence
  Synthetic
  misc_feature (1)..(13): deoxyribonucleoside with tricyclic sugar
  misc_feature (1)..(12): phosphorothioate internucleoside linkage group between the 3' end of this nucleoside and the 5' end of the next nucleoside
  modified_base (1)..(2): m5c
  modified_base (4)..(4): m5c
  modified_base (7)..(7): m5c
  modified_base (11)..(12): m5c
cctcggcttacct

SEQ ID NO: 24 - DNA, 15 bp, Artificial Sequence
  Synthetic
  misc_feature (1)..(4): deoxyribonucleoside with tricyclic sugar
  misc_feature (1)..(1): a phosphorothioate internucleoside linkage group between the 3' end of this nucleoside and the 5' end of the next nucleoside
  misc_feature (5)..(5): 2'-modified ribonucleoside, preferably 2'-O-methyl ribonucleoside
  misc_feature (6)..(15): deoxyribonucleoside with tricyclic sugar
  modified_base (8)..(8): m5c
  modified_base (13)..(13): m5c
aagauggcatttcta

SEQ ID NO: 25 - DNA, 15 bp, Artificial Sequence
  Synthetic
  misc_feature (1)..(4): deoxyribonucleoside with tricyclic sugar
  misc_feature (1)..(2): a phosphorothioate internucleoside linkage group between the 3' end of this nucleoside and the 5' end of the next nucleoside
  misc_feature (5)..(5): 2'-modified ribonucleoside, preferably 2'-O-methyl ribonucleoside
  misc_feature (6)..(15): deoxyribonucleoside with tricyclic sugar
  modified_base (8)..(8): m5c
  modified_base (13)..(13): m5c
aagauggcatttcta

SEQ ID NO: 26 - DNA, 15 bp, Artificial Sequence
  Synthetic
  misc_feature (1)..(4): deoxyribonucleoside with tricyclic sugar
  misc_feature (1)..(3): a phosphorothioate internucleoside linkage group between the 3' end of this nucleoside and the 5' end of the next nucleoside
  misc_feature (5)..(5): 2'-modified ribonucleoside, preferably 2'-O-methyl ribonucleoside
  misc_feature (6)..(15): deoxyribonucleoside with tricyclic sugar
  modified_base (8)..(8): m5c
  modified_base (13)..(13): m5c
aagauggcatttcta

SEQ ID NO: 27 - DNA, 15 bp, Artificial Sequence
  Synthetic
  misc_feature (1)..(4): deoxyribonucleoside with tricyclic sugar
  misc_feature (1)..(4): a phosphorothioate internucleoside linkage group between the 3' end of this nucleoside and the 5' end of the next nucleoside
  misc_feature (5)..(5): 2'-modified ribonucleoside, preferably 2'-O-methyl ribonucleoside
  misc_feature (6)..(15): deoxyribonucleoside with tricyclic sugar
  modified_base (8)..(8): m5c
  modified_base (13)..(13): m5c
aagauggcatttcta

SEQ ID NO: 28 - DNA, 15 bp, Artificial Sequence
  Synthetic
  misc_feature (1)..(4): deoxyribonucleoside with tricyclic sugar
  misc_feature (1)..(5): a phosphorothioate internucleoside linkage group between the 3' end of this nucleoside and the 5' end of the next nucleoside
  misc_feature (5)..(5): 2'-modified ribonucleoside, preferably 2'-O-methyl ribonucleoside
  misc_feature (6)..(15): deoxyribonucleoside with tricyclic sugar
  modified_base (8)..(8): m5c
  modified_base (13)..(13): m5c
aagauggcatttcta

SEQ ID NO: 29 - DNA, 15 bp, Artificial Sequence
  Synthetic
  misc_feature (1)..(4): deoxyribonucleoside with tricyclic sugar
  misc_feature (1)..(6): a phosphorothioate internucleoside linkage group between the 3' end of this nucleoside and the 5' end of the next nucleoside
  misc_feature (5)..(5): 2'-modified ribonucleoside, preferably 2'-O-methyl ribonucleoside
  misc_feature (6)..(15): deoxyribonucleoside with tricyclic sugar
  modified_base (8)..(8): m5c
  modified_base (13)..(13): m5c
aagauggcatttcta

SEQ ID NO: 30 - DNA, 15 bp, Artificial Sequence
  Synthetic
  misc_feature (1)..(4): deoxyribonucleoside with tricyclic sugar
  misc_feature (1)..(7): a phosphorothioate internucleoside linkage group between the 3' end of this nucleoside and the 5' end of the next nucleoside
  misc_feature (5)..(5): 2'-modified ribonucleoside, preferably 2'-O-methyl ribonucleoside
  misc_feature (6)..(15): deoxyribonucleoside with tricyclic sugar
  modified_base (8)..(8): m5c
  modified_base (13)..(13): m5c
aagauggcatttcta

SEQ ID NO: 31 - DNA, 15 bp, Artificial Sequence
  Synthetic
  misc_feature (1)..(15): deoxyribonucleoside with tricyclic sugar
  misc_feature (1)..(1): a phosphorothioate internucleoside linkage group between the 3' end of this nucleoside and the 5' end of the next nucleoside
  modified_base (8)..(8): m5c
  modified_base (13)..(13): m5c
aagatggcatttcta

SEQ ID NO: 32 - DNA, 15 bp, Artificial Sequence
  Synthetic
  misc_feature (1)..(15): deoxyribonucleoside with tricyclic sugar
  misc_feature (1)..(2): a phosphorothioate internucleoside linkage group between the 3' end of this nucleoside and the 5' end of the next nucleoside
  modified_base (8)..(8): m5c
  modified_base (13)..(13): m5c
aagatggcatttcta

SEQ ID NO: 33 - DNA, 15 bp, Artificial Sequence
  Synthetic
  misc_feature (1)..(15): deoxyribonucleoside with tricyclic sugar
  misc_feature (1)..(3): a phosphorothioate internucleoside linkage group between the 3' end of this nucleoside and the 5' end of the next nucleoside
  modified_base (8)..(8): m5c
  modified_base (13)..(13): m5c
aagatggcatttcta

SEQ ID NO: 34 - DNA, 15 bp, Artificial Sequence
  Synthetic
  misc_feature (1)..(15): deoxyribonucleoside with tricyclic sugar
  misc_feature (1)..(4): a phosphorothioate internucleoside linkage group between the 3' end of this nucleoside and the 5' end of the next nucleoside
  modified_base (8)..(8): m5c
  modified_base (13)..(13): m5c
aagatggcatttcta

SEQ ID NO: 35 - DNA, 15 bp, Artificial Sequence
  Synthetic
  misc_feature (1)..(15): deoxyribonucleoside with tricyclic sugar
  misc_feature (1)..(5): a phosphorothioate internucleoside linkage group between the 3' end of this nucleoside and the 5' end of the next nucleoside
  modified_base (8)..(8): m5c
  modified_base (13)..(13): m5c
aagatggcatttcta

SEQ ID NO: 36 - DNA, 15 bp, Artificial Sequence
  Synthetic
  misc_feature (1)..(15): deoxyribonucleoside with tricyclic sugar
  misc_feature (1)..(6): a phosphorothioate internucleoside linkage group between the 3' end of this nucleoside and the 5' end of the next nucleoside
  modified_base (8)..(8): m5c
  modified_base (13)..(13): m5c
aagatggcatttcta

SEQ ID NO: 37 - DNA, 15 bp, Artificial Sequence
  Synthetic
  misc_feature (1)..(15): deoxyribonucleoside with tricyclic sugar
  misc_feature (1)..(7): a phosphorothioate internucleoside linkage group between the 3' end of this nucleoside and the 5' end of the next nucleoside
  modified_base (8)..(8): m5c
  modified_base (13)..(13): m5c
aagatggcatttcta

SEQ ID NO: 38 - DNA, 22 bp, Artificial Sequence
  Synthetic
cagaattctgccaattgctgag

SEQ ID NO: 39 - DNA, 20 bp, Artificial Sequence
  Synthetic
ttcttcagcttgtgtcatcc

SEQ ID NO: 40 - DNA, 24 bp, Artificial Sequence
  Synthetic
cccagtctaccaccctatcagagc

SEQ ID NO: 41 - DNA, 20 bp, Artificial Sequence
  Synthetic
cctgcctttaaggcttcctt

SEQ ID NO: 42 - DNA, 13 bp, Artificial Sequence
  Synthetic
  misc_feature (1)..(13): deoxyribonucleoside with tricyclic sugar
  misc_feature (1)..(1): terminal phosphate group
  misc_feature (10)..(12): phosphorothioate internucleoside linkage group between the 3' end of this nucleoside and the 5' end of the next nucleoside
cctcggcttacct

SEQ ID NO: 43 - DNA, 13 bp, Artificial Sequence
  Synthetic
  misc_feature (1)..(13): deoxyribonucleoside with tricyclic sugar
  misc_feature (1)..(1): terminal phosphate group
  misc_feature (9)..(12): phosphorothioate internucleoside linkage group between the 3' end of this nucleoside and the 5' end of the next nucleoside
cctcggcttacct

SEQ ID NO: 44 - DNA, 13 bp, Artificial Sequence
  Synthetic
  misc_feature (1)..(1): terminal phosphate group
  misc_feature (1)..(13): deoxyribonucleoside with tricyclic sugar
  misc_feature (7)..(12): phosphorothioate internucleoside linkage group between the 3' end of this nucleoside and the 5' end of the next nucleoside
cctcggcttacct

SEQ ID NO: 45 - DNA, 13 bp, Artificial Sequence
  Synthetic
  misc_feature (1)..(13): deoxyribonucleoside with tricyclic sugar
  misc_feature (1)..(1): terminal phosphate group
  misc_feature (5)..(12): phosphorothioate internucleoside linkage group between the 3' end of this nucleoside and the 5' end of the next nucleoside
cctcggcttacct

SEQ ID NO: 46 - DNA, 13 bp, Artificial Sequence
  Synthetic
  misc_feature (1)..(13): deoxyribonucleoside with tricyclic sugar
  misc_feature (1)..(1): terminal phosphate group
  misc_feature (3)..(12): phosphorothioate internucleoside linkage group between the 3' end of this nucleoside and the 5' end of the next nucleoside
cctcggcttacct

SEQ ID NO: 47 - DNA, 15 bp, Artificial Sequence
  Synthetic
  misc_feature (1)..(15): deoxyribonucleoside with tricyclic sugar
ctttcataatgctgg